European Patent Application EP 4 438 616 A1, published October 2, 2024. Title: NEW POLYPEPTIDE FOR PROMOTING TISSUE REPAIR, AND USE THEREOF. Applicant: Jinan University. The sequence listing filed with the application follows.

SEQUENCE LISTING (12 sequences)

SEQ ID NO: 1 - protein, 9 aa, Artificial Sequence
  NEW POLYPEPTIDE TRF1 FOR PROMOTING TISSUE REPAIR
  DISULFID (2)..(8)
ACPNYPYCY

SEQ ID NO: 2 - protein, 10 aa, Artificial Sequence
  NEW POLYPEPTIDE TRF2 FOR PROMOTING TISSUE REPAIR
  DISULFID (3)..(9)
AACPNYPYCY

SEQ ID NO: 3 - protein, 11 aa, Artificial Sequence
  NEW POLYPEPTIDE TRF3 FOR PROMOTING TISSUE REPAIR
  DISULFID (4)..(10)
AAACPNYPYCY

SEQ ID NO: 4 - protein, 11 aa, Artificial Sequence
  NEW POLYPEPTIDE TRF4 FOR PROMOTING TISSUE REPAIR
  DISULFID (4)..(10)
VAACPDYPYCS

SEQ ID NO: 5 - protein, 11 aa, Artificial Sequence
  NEW POLYPEPTIDE TRF5 FOR PROMOTING TISSUE REPAIR
  DISULFID (4)..(10)
AAACPDYPYCS

SEQ ID NO: 6 - protein, 19 aa, Artificial Sequence
  NEW POLYPEPTIDE TRF6 FOR PROMOTING TISSUE REPAIR
  DISULFID (2)..(8)
ACPNYPYCGSYAPLGYHVR

SEQ ID NO: 7 - protein, 28 aa, Artificial Sequence
  NEW POLYPEPTIDE TRF7 FOR PROMOTING TISSUE REPAIR
  DISULFID (2)..(8)
ACPNYPYCGSYAPLGYHVREYPAGVSAA

SEQ ID NO: 8 - protein, 10 aa, Artificial Sequence
  NEW POLYPEPTIDE TRF8 FOR PROMOTING TISSUE REPAIR
  DISULFID (3)..(9)
AACPDYPYCS

SEQ ID NO: 9 - protein, 10 aa, Artificial Sequence
  NEW POLYPEPTIDE TRF9 FOR PROMOTING TISSUE REPAIR
  DISULFID (3)..(9)
GACPDYPYCY

SEQ ID NO: 10 - protein, 11 aa, Artificial Sequence
  NEW POLYPEPTIDE TRF10 FOR PROMOTING TISSUE REPAIR
  DISULFID (4)..(10)
AAACPDYPYCY

SEQ ID NO: 11 - protein, 11 aa, Artificial Sequence
  NEW POLYPEPTIDE TRF11 FOR PROMOTING TISSUE REPAIR
  DISULFID (2)..(8)
ACPNYPYCGSY

SEQ ID NO: 12 - protein, 16 aa, Artificial Sequence
  NEW POLYPEPTIDE TRF12 FOR PROMOTING TISSUE REPAIR
  DISULFID (2)..(8)
ACPNYPYCGSYAPLGY